European Patent Specification EP 4 050 101 B1, published June 26, 2024. Title: Novel phytoene synthase variant and a method for producing XMP or GMP using the same. Applicant: CJ CheilJedang Corporation. The sequence listing filed with the application follows.

SEQUENCE LISTING (11 sequences)

SEQ ID NO: 1 - protein, 283 aa, Artificial Sequence
  CRTB2_A133V
MNSPTRRALIETYDKTARRASGKIISGYSSSFSLATRLLAEPARTDIRHLYAVVRIADEIVDGTALEVGANPAKLLNEYEEQVRKAAEQKFHTDPVMHAFAMTARRCNFKDEHLRAFFTSMRRDLDSSAHDAVSFDSYVYGSAEVIGLLCLDVFLADRKTGAKEREQLDAGARHLGAAFQKINFLRDRHEDFEILGREYFPEGTTLEAILSDIRDDIEIARTVIPGLPLRARAGVLAATGIFEELTSQLADSRSDKTRISVPRRKKLGIAVRAAVTALKGNNK

SEQ ID NO: 2 - DNA, 852 bp, Artificial Sequence
  crtB2_C398T
atgaattcacccacgaggcgcgcgctgattgagacctacgataagactgctcgtcgtgcgtctggcaaaattatctcgggatattcctccagtttctcgcttgcaacgcgcctgctagctgaacccgcccgaacagatatccgccatctttacgcagttgtccgtatagcggacgaaattgtcgatggcactgcacttgaagtcggcgccaatccggccaagctactcaacgagtacgaggaacaggttcgaaaggcagcagaacaaaaatttcatacggaccctgtcatgcatgcttttgccatgactgcacggcgctgcaatttcaaagacgagcacctcagagcatttttcacatccatgcgccgcgacttggattcctccgctcatgatgctgttagctttgattcatatgtctacggctcagcggaagtcattggattgctgtgcctggatgtgtttctcgcagatagaaaaactggcgcgaaggaaagagaacagctcgatgcaggagcaagacaccttggtgccgcgtttcagaagatcaatttccttagagaccggcacgaagattttgaaatcctaggaagagagtactttcccgagggaactactctcgaagctattctgtccgatatccgagatgacatcgaaatcgctcggaccgtcatcccggggcttcctttgagagctcgagcaggagtattagctgcgaccggcatattcgaagaactaacatcacaattggcagatagccgatcggataagacgcgaattagtgttccacgccggaagaagctcggaattgcggtacgcgcagctgtgacagcattgaaagggaacaataagtga

SEQ ID NO: 3 - protein, 283 aa, Artificial Sequence
  CRTB2
MNSPTRRALIETYDKTARRASGKIISGYSSSFSLATRLLAEPARTDIRHLYAVVRIADEIVDGTALEVGANPAKLLNEYEEQVRKAAEQKFHTDPVMHAFAMTARRCNFKDEHLRAFFTSMRRDLDSSAHDAASFDSYVYGSAEVIGLLCLDVFLADRKTGAKEREQLDAGARHLGAAFQKINFLRDRHEDFEILGREYFPEGTTLEAILSDIRDDIEIARTVIPGLPLRARAGVLAATGIFEELTSQLADSRSDKTRISVPRRKKLGIAVRAAVTALKGNNK

SEQ ID NO: 4 - DNA, 852 bp, Artificial Sequence
  crtB2
atgaattcacccacgaggcgcgcgctgattgagacctacgataagactgctcgtcgtgcgtctggcaaaattatctcgggatattcctccagtttctcgcttgcaacgcgcctgctagctgaacccgcccgaacagatatccgccatctttacgcagttgtccgtatagcggacgaaattgtcgatggcactgcacttgaagtcggcgccaatccggccaagctactcaacgagtacgaggaacaggttcgaaaggcagcagaacaaaaatttcatacggaccctgtcatgcatgcttttgccatgactgcacggcgctgcaatttcaaagacgagcacctcagagcatttttcacatccatgcgccgcgacttggattcctccgctcatgatgctgctagctttgattcatatgtctacggctcagcggaagtcattggattgctgtgcctggatgtgtttctcgcagatagaaaaactggcgcgaaggaaagagaacagctcgatgcaggagcaagacaccttggtgccgcgtttcagaagatcaatttccttagagaccggcacgaagattttgaaatcctaggaagagagtactttcccgagggaactactctcgaagctattctgtccgatatccgagatgacatcgaaatcgctcggaccgtcatcccggggcttcctttgagagctcgagcaggagtattagctgcgaccggcatattcgaagaactaacatcacaattggcagatagccgatcggataagacgcgaattagtgttccacgccggaagaagctcggaattgcggtacgcgcagctgtgacagcattgaaagggaacaataagtga

SEQ ID NO: 5 - DNA, 35 bp, Artificial Sequence
  Primer
tcgagctcggtacccgtgaggatgcctaaccgaaa

SEQ ID NO: 6 - DNA, 41 bp, Artificial Sequence
  Primer
catatgaatcaaagctaacagcatcatgagcggaggaatcc

SEQ ID NO: 7 - DNA, 41 bp, Artificial Sequence
  Primer
ggattcctccgctcatgatgctgttagctttgattcatatg

SEQ ID NO: 8 - DNA, 35 bp, Artificial Sequence
  Primer
ctctagaggatcccctgttccctttcaatgctgtc

SEQ ID NO: 9 - DNA, 20 bp, Artificial Sequence
  Primer-5F
gtgaggatgcctaaccgaaa

SEQ ID NO: 10 - DNA, 20 bp, Artificial Sequence
  Primer
tgttccctttcaatgctgtc

SEQ ID NO: 11 - DNA, 5803 bp, Artificial Sequence
  pDCM2
gttcgcttgctgtccataaaaccgcccagtctagctatcgccatgtaagcccactgcaagctacctgctttctctttgcgcttgcgttttcccttgtccagatagcccagtagctgacattcatccggggtcagcaccgtttctgcggactggctttctacgtgttccgcttcctttagcagcccttgcgccctgagtgcttgcggcagcgtgaagctagcttttatcgccattcgccattcaggctgcgcaactgttgggaagggcgatcggtgcgggcctcttcgctattacgccagctggcgaaagggggatgtgctgcaaggcgattaagttgggtaacgccagggttttcccagtcacgacgttgtaaaacgacggccagtgaattcgagctcggtacccggggatcctctagagtcgacctgcaggcatgcaagcttggcgtaatcatggtcatagctgtttcctgtgtgaaattgttatccgctcacaattccacacaacatacgagccggaagcataaagtgtaaagcctggggtgcctaatgagtgagctaactcacattaattgcgttgcgctcactgcccgctttccagtcgggaaacctgtcgtgccagctgcattaatgaatcggccaacgcgcggggagaggcggtttgcgtattgggcgctcttccgcttcctcgctcactgactcgctgcgctcggtcgttcggctgcggcgagcggtatcagctcactcaaaggcggtaatacggttatccacagaatcaggggataacgcaggaaagaacatgtgagcaaaaggccagcaaaaggccaggaaccgtaaaaaggccgcgttgctggcgtttttccataggctccgcccccctgacgagcatcacaaaaatcgacgctcaagtcagaggtggcgaaacccgacaggactataaagataccaggcgtttccccctggaagctccctcgtgcgctctcctgttccgaccctgccgcttaccggatacctgtccgcctttctcccttcgggaagcgtggcgctttctcaatgctcacgctgtaggtatctcagttcggtgtaggtcgttcgctccaagctgggctgtgtgcacgaaccccccgttcagcccgaccgctgcgccttatccggtaactatcgtcttgagtccaacccggtaagacacgacttatcgccactggcagcagccactggtaacaggattagcagagcgaggtatgtaggcggtgctacagagttcttgaagtggtggcctaactacggctacactagaaggacagtatttggtatctgcgctctgctgaagccagttaccttcggaaaaagagttggtagctcttgatccggcaaacaaaccaccgctggtagcggtggtttttttgtttgcaagcagcagattacgcgcagaaaaaaaggatctcaagaagatcctttgatcttttctacggggtctgacgctcagtggaacgaaaactcacgttaagggattttggtcatgagattatcaaaaaggatcttcacctagatccttttggggtgggcgaagaactccagcatgagatccccgcgctggaggatcatccagccctgatagaaacagaagccactggagcacctcaaaaacaccatcatacactaaatcagtaagttggcagcatcacccgacgcactttgcgccgaataaatacctgtgacggaagatcacttcgcagaataaataaatcctggtgtccctgttgataccgggaagccctgggccaacttttggcgaaaatgagacgttgatcggcacgtaagaggttccaactttcaccataatgaaataagatcactaccgggcgtattttttgagttatcgagattttcaggagctgatagaaacagaagccactggagcacctcaaaaacaccatcatacactaaatcagtaagttggcagcatcacccgacgcactttgcgccgaataaatacctgtgacggaagatcacttcgcagaataaataaatcctggtgtccctgttgataccgggaagccctgggccaacttttggcgaaaatgagacgttgatcggcacgtaagaggttccaactttcaccataatgaaataagatcactaccgggcgtattttttgagttatcgagattttcaggagctctttggcatcgtctctcgcctgtcccctcagttcagtaatttcctgcatttgcctgtttccagtcggtagatattccacaaaacagcagggaagcagcgcttttccgctgcataaccctgcttcggggtcattatagcgattttttcggtatatccatcctttttcgcacgatatacaggattttgccaaagggttcgtgtagactttccttggtgtatccaacggcgtcagccgggcaggataggtgaagtaggcccacccgcgagcgggtgttccttcttcactgtcccttattcgcacctggcggtgctcaacgggaatcctgctctgcgaggctggccggctaccgccggcgtaacagatgagggcaagcggatggctgatgaaaccaagccaaccaggaagggcagcccacctatcaaggtgtactgccttccagacgaacgaagagcgattgaggaaaaggcggcggcggccggcatgagcctgtcggcctacctgctggccgtcggccagggctacaaaatcacgggcgtcgtggactatgagcacgtccgcgagggcgtcccggaaaacgattccgaagcccaacctttcatagaaggcggcggtggaatcgaaatctcgtgatggcaggttgggcgtcgcttggtcggtcatttcgaaaaaggttaggaatacggttagccatttgcctgcttttatatagttcantatgggattcacctttatgttgataagaaataaaagaaaatgccaataggatatcggcattttcttttgcgtttttatttgttaactgttaattgtccttgttcaaggatgctgtctttgacaacagatgttttcttgcctttgatgttcagcaggaagctcggcgcaaacgttgattgtttgtctgcgtagaatcctctgtttgtcatatagcttgtaatcacgacattgtttcctttcgcttgaggtacagcgaagtgtgagtaagtaaaggttacatcgttaggcggatcaagatccatttttaacacaaggccagttttgttcagcggcttgtatgggccagttaaagaattagaaacataaccaagcatgtaaatatcgttagacgtaatgccgtcaatcgtcatttttgatccgcgggagtcagtgaacaggtaccatttgccgttcattttaaagacgttcgcgcgttcaatttcatctgttactgtgttagatgcaatcagcggtttcatcacttttttcagtgtgtaatcatcgtttagctcaatcataccgagagcgccgtttgctaactcagccgtgcgttttttatcgctttgcagaagtttttgactttcttgacggaagaatgatgtgcttttgccatagtatgctttgttaaataaagattcttcgccttggtagccatcttcagttccagtgtttgcttcaaatactaagtatttgtggcctttatcttctacgtagtgaggatctctcagcgtatggttgtcgcctgagctgtagttgccttcatcgatgaactgctgtacattttgatacgtttttccgtcaccgtcaaagattgatttataatcctctacaccgttgatgttcaaagagctgtctgatgctgatacgttaacttgtgcagttgtcagtgtttgtttgccgtaatgtttaccggagaaatcagtgtagaataaacggatttttccgtcagatgtaaatgtggctgaacctgaccattcttgtgtttggtcttttaggatagaatcatttgcatcgaatttgtcgctgtctttaaagacgcggccagcgtttttccagctgtcaatagaagtttcgccgactttttgatagaacatgtaaatcgatgtgtcatccgcatttttaggatctccggctaatgcaaagacgatgtggtagccgtgatagtttgcgacagtgccgtcagcgttttgtaatggccagctgtcccaaacgtccaggccttttgcagaagagatatttttaattgtggacgaatcaaattcagaaacttgatatttttcatttttttgctgttcagggatttgcagcatatcatggcgtgtaatatgggaaatgccgtatgtttccttatatggcttttggttcgtttctttcgcaaacgcttgagttgcgcctcctgccagcagtgcggtagtaaaggttaatactgttgcttgttttgcaaactttttgatgttcatcgttcatgtctccttttttatgtactgtgttagcggtctgcttcttccagccctcctgtttgaagatggcaagttagttacgcacaataaaaaaagacctaaaatatgtaaggggtgacgccaaagtatacactttgccctttacacattttaggtcttgcctgctttatcagtaacaaacccgcgcgatttacttttcgacctcattctattagactctcgtttggattgcaactggtctattttcctcttttgtttgatagaaaatcataaaaggatttgcagactacgggcctaaagaactaaaaaatctatctgtttcttttcattctctgtattttttatagtttctgttgcatgggcataaagttgcctttttaatcacaattcagaaaatatcataatatctcatttcactaaataatagtgaacggcaggtatatgtgatgggttaaaaaggatcaccccagagtcccgctcagaagaactcgtcaagaaggcgatagaaggcgatgcgctgcgaatcgggagcggcgataccgtaaagcacgaggaagcggtcagcccattcgccgccaagctcttcagcaatatcacgggtagccaacgctatgtcctgatagcggtccgccacacccagccggccacagtcgatgaatccagaaaagcggccattttccaccatgatattcggcaagcaggcatcgccatgggtcacgacgagatcctcgccgtcgggcatccgcgccttgagcctggcgaacagttcggctggcgcgagcccctgatgctcttcgtccagatcatcctgatcgacaagaccggcttccatccgagtacgtgctcgctcgatgcgatgtttcgcttggtggtcgaatgggcaggtagccggatcaagcgtatgcagccgccgcattgcatcagccatgatggatactttctcggcaggagcaaggtgagatgacaggagatcctgccccggcacttcgcccaatagcagccagtcccttcccgcttcagtgacaacgtcgagacagctgcgcaaggaacgcccgtcgtggccagccacgatagccgcgctgcctcgtcttggagttcattcagggcaccggacaggtcggtcttgacaaaaagaaccgggcgcccctgcgctgacagccggaacacggcggcatcagagcagccgattgtctgttgtgcccagtcatagccgaatagcctctccacccaagcggccggagaacctgcgtgcaatccatcttgttcaatcatgcgaaacgatcctcatcctgtctcttgatcagatcttgatcccctgcgccatcagatccttggcggcaagaaagccatccagtttactttgcagggcttcccaaccttaccagagggcgccccagctggcaattccg